European Patent Specification EP 3 450 569 B1, published May 13, 2026. Title: DNA AMPLIFICATION METHOD. Applicant: Xukang (Suzhou) Medical Science & Technology Co.,Ltd. Application EP17788769.2. The sequence listing filed with the application follows.

SEQUENCE LISTING (42 sequences)

SEQ ID NO: 1 - DNA, 13 bp, Artificial sequence
  Synthetic
ttggtagtgagtg

SEQ ID NO: 2 - DNA, 13 bp, Artificial sequence
  Synthetic
gaggtgtgatgga

SEQ ID NO: 3 - DNA, 15 bp, Artificial sequence
  Synthetic
gtgatggttgaggta

SEQ ID NO: 4 - DNA, 19 bp, Artificial sequence
  Synthetic
agatgtgtataagagacag

SEQ ID NO: 5 - DNA, 27 bp, Artificial sequence
  Synthetic
gtgagtgatggttgaggtagtgtggag

SEQ ID NO: 6 - DNA, 13 bp, Artificial sequence
  Synthetic
gctcttccgatct

SEQ ID NO: 7 - DNA, 23 bp, Artificial sequence
  Synthetic
  misc_feature (14)..(14): N = A or T or C or G
  misc_feature (15)..(19): B = T or C or G
gctcttccgatctnbbbbbtggg

SEQ ID NO: 8 - DNA, 23 bp, Artificial sequence
  Synthetic
  misc_feature (14)..(14): N = A or T or C or G
  misc_feature (15)..(19): D = A or T or G
gctcttccgatctndddddtggg

SEQ ID NO: 9 - DNA, 23 bp, Artificial sequence
  Synthetic
  misc_feature (14)..(14): N = A or T or C or G
  misc_feature (15)..(19): H = A or T or C
gctcttccgatctnhhhhhtggg

SEQ ID NO: 10 - DNA, 23 bp, Artificial sequence
  Synthetic
  misc_feature (14)..(14): N = A or T or C or G
  misc_feature (15)..(19): V = A or C or G
gctcttccgatctnvvvvvtggg

SEQ ID NO: 11 - DNA, 23 bp, Artificial sequence
  Synthetic
  misc_feature (14)..(14): N = A or T or C or G
  misc_feature (15)..(19): B = T or C or G
gctcttccgatctnbbbbbgttt

SEQ ID NO: 12 - DNA, 23 bp, Artificial sequence
  Synthetic
  misc_feature (14)..(14): N = A or T or C or G
  misc_feature (15)..(19): D = A or T or G
gctcttccgatctndddddgttt

SEQ ID NO: 13 - DNA, 23 bp, Artificial sequence
  Synthetic
  misc_feature (14)..(14): N = A or T or C or G
  misc_feature (14)..(14): H = A or T or C
gctcttccgatctnhhhhhgttt

SEQ ID NO: 14 - DNA, 23 bp, Artificial sequence
  Synthetic
  misc_feature (14)..(14): N = A or T or C or G
  misc_feature (15)..(19): V = A or C or G
gctcttccgatctnvvvvvgttt

SEQ ID NO: 15 - DNA, 23 bp, Artificial sequence
  Synthetic
  misc_feature (14)..(14): N = A or T or C or G
  misc_feature (15)..(19): B = T or C or G
ttggtagtgagtgnbbbbbtggg

SEQ ID NO: 16 - DNA, 23 bp, Artificial sequence
  Synthetic
  misc_feature (14)..(14): N = A or T or C or G
  misc_feature (15)..(19): D = A or T or G
ttggtagtgagtgndddddtggg

SEQ ID NO: 17 - DNA, 23 bp, Artificial sequence
  Synthetic
  misc_feature (14)..(14): N = A or T or C or G
  misc_feature (15)..(19): H = A or T or C
ttggtagtgagtgnhhhhhtggg

SEQ ID NO: 18 - DNA, 23 bp, Artificial sequence
  Synthetic
  misc_feature (14)..(14): N = A or T or C or G
  misc_feature (15)..(19): V = A or C or G
ttggtagtgagtgnvvvvvtggg

SEQ ID NO: 19 - DNA, 23 bp, Artificial sequence
  Synthetic
  misc_feature (14)..(14): N = A or T or C or G
  misc_feature (15)..(19): B = T or C or G
ttggtagtgagtgnbbbbbgttt

SEQ ID NO: 20 - DNA, 23 bp, Artificial sequence
  Synthetic
  misc_feature (14)..(14): N = A or T or C or G
  misc_feature (15)..(19): D = A or T or G
ttggtagtgagtgndddddgttt

SEQ ID NO: 21 - DNA, 23 bp, Artificial sequence
  Synthetic
  misc_feature (14)..(14): N = A or T or C or G
  misc_feature (15)..(19): H = A or T or C
ttggtagtgagtgnhhhhhgttt

SEQ ID NO: 22 - DNA, 23 bp, Artificial sequence
  Synthetic
  misc_feature (14)..(14): N = A or T or C or G
  misc_feature (15)..(19): V = A or C or G
ttggtagtgagtgnvvvvvgttt

SEQ ID NO: 23 - DNA, 23 bp, Artificial sequence
  Synthetic
  misc_feature (14)..(14): N = A or T or C or G
  misc_feature (15)..(19): B = T or C or G
gaggtgtgatgganbbbbbtggg

SEQ ID NO: 24 - DNA, 23 bp, Artificial sequence
  Synthetic
  misc_feature (14)..(14): N = A or T or C or G
  misc_feature (15)..(19): D = A or T or G
gaggtgtgatggandddddtggg

SEQ ID NO: 25 - DNA, 23 bp, Artificial sequence
  Synthetic
  misc_feature (14)..(14): N = A or T or C or G
  misc_feature (15)..(19): H = A or T or C
gaggtgtgatgganhhhhhtggg

SEQ ID NO: 26 - DNA, 23 bp, Artificial sequence
  Synthetic
  misc_feature (14)..(14): N = A or T or C or G
  misc_feature (15)..(19): V = A or C or G
gaggtgtgatgganvvvvvtggg

SEQ ID NO: 27 - DNA, 23 bp, Artificial sequence
  Synthetic
  misc_feature (14)..(14): N = A or T or C or G
  misc_feature (15)..(19): B = T or C or G
gaggtgtgatgganbbbbbgttt

SEQ ID NO: 28 - DNA, 24 bp, Artificial sequence
  Synthetic
  misc_feature (14)..(14): N = A or T or C or G
  misc_feature (15)..(19): D = A or T or G
gaggtgtgatgganddddddgttt

SEQ ID NO: 29 - DNA, 23 bp, Artificial sequence
  Synthetic
  misc_feature (14)..(14): N = A or T or C or G
  misc_feature (15)..(19): H = A or T or C
gaggtgtgatgganhhhhhgttt

SEQ ID NO: 30 - DNA, 23 bp, Artificial sequence
  Synthetic
  misc_feature (14)..(14): N = A or T or C or G
  misc_feature (15)..(19): V = A or C or G
gaggtgtgatgganvvvvvgttt

SEQ ID NO: 31 - DNA, 20 bp, Artificial sequence
  Synthetic
acactctttccctacacgac

SEQ ID NO: 32 - DNA, 21 bp, Artificial sequence
  Synthetic
gtgactggagttcagacgtgt

SEQ ID NO: 33 - DNA, 25 bp, Artificial sequence
  Synthetic
aatgatacggcgaccaccgagatct

SEQ ID NO: 34 - DNA, 24 bp, Artificial sequence
  Synthetic
caagcagaagacggcatacgagat

SEQ ID NO: 35 - DNA, 58 bp, Artificial sequence
  Synthetic
aatgatacggcgaccaccgagatctacactctttccctacacgacgctcttccgatct

SEQ ID NO: 36 - DNA, 64 bp, Artificial sequence
  Synthetic
  misc_feature: Barcode sequence
caagcagaagacggcatacgagatcgtgatgtgactggagttcagacgtgtgctcttccgatct

SEQ ID NO: 37 - DNA, 54 bp, Artificial sequence
  Synthetic
ccactacgcctccgctttcctctctatgggcagtcggtgatgctcttccgatct

SEQ ID NO: 38 - DNA, 54 bp, Artificial sequence
  Synthetic
  misc_feature (31)..(40): Barcode sequence
ccactacgcctccgctttcctctctatgggcagtcggtgatttggtagtgagtg

SEQ ID NO: 39 - DNA, 56 bp, Artificial sequence
  Synthetic
ccatctcatccctgcgtgtctccgactcagctaaggtaacgatttggtagtgagtg

SEQ ID NO: 40 - DNA, 56 bp, Artificial sequence; identical to SEQ ID NO: 39
  Synthetic
  misc_feature: Barcode sequence

SEQ ID NO: 41 - DNA, 54 bp, Artificial sequence
  Synthetic
ccactacgcctccgctttcctctctatgggcagtcggtgatgaggtgtgatgga

SEQ ID NO: 42 - DNA, 56 bp, Artificial sequence
  Synthetic
  misc_feature (31)..(40): Barcode sequence
ccatctcatccctgcgtgtctccgactcagctaaggtaacgatgaggtgtgatgga